European Patent Application EP 4 772 681 A1, published July 8, 2026. Title: 一种空间条形码芯片的制备方法及其应用. Applicant: 北京寻因生物科技有限公司. The sequence listing filed with the application follows.

SEQUENCE LISTING (8 sequences)

SEQ ID NO: 1 - DNA, 113 bp, synthetic construct
  source 1..113: mol_type = other DNA
aatgatacggcgaccaccgagatctacacgtgactggagttcagacgtgtgctcttccgatctnnnnnnnnnnnnnnnnnnnnnnnnnnnnnnnntcttgtgactacagcacc

SEQ ID NO: 2 - DNA, 74 bp, synthetic construct
  source 1..74: mol_type = other DNA
  modified_base 1: mod_base = OTHER; note = phosphorylated guanosine
gactttcaccagtccatgataaaaaaaaaaaaaaaaaaaaaaaaaaaaaaatctcgtatgccgtcttctgcttg

SEQ ID NO: 3 - DNA, 21 bp, synthetic construct
  source 1..21: mol_type = other DNA
ggtgaaagtcggtgctgtagt

SEQ ID NO: 4 - DNA, 187 bp, synthetic construct
  source 1..187: mol_type = other DNA
aatgatacggcgaccaccgagatctacacgtgactggagttcagacgtgtgctcttccgatctnnnnnnnnnnnnnnnnnnnnnnnnnnnnnnnntcttgtgactacagcaccgactttcaccagtccatgataaaaaaaaaaaaaaaaaaaaaaaaaaaaaaatctcgtatgccgtcttctgcttg

SEQ ID NO: 5 - DNA, 29 bp, synthetic construct
  source 1..29: mol_type = other DNA
aatgatacggcgaccaccgagatctacac

SEQ ID NO: 6 - DNA, 34 bp, synthetic construct
  source 1..34: mol_type = other DNA
gtgactggagttcagacgtgtgctcttccgatct

SEQ ID NO: 7 - DNA, 38 bp, synthetic construct
  source 1..38: mol_type = other DNA
tcttgtgactacagcaccgactttcaccagtccatgat

SEQ ID NO: 8 - DNA, 24 bp, synthetic construct
  source 1..24: mol_type = other DNA
atctcgtatgccgtcttctgcttg